European Patent Specification EP 3 377 091 B1, published September 20, 2023. Title: Secreted splicing variant of mammal Klotho as a medicament for cognition and behaviour impairments. Applicant: UNIVERSITAT AUTñNOMA DE BARCELONA. The sequence listing filed with the application follows.

SEQUENCE LISTING (19 sequences)

SEQ ID NO: 1 - protein, 549 aa, Homo sapiens
MPASAPPRRPRPPPPSLSLLLVLLGLGGRRLRAEPGDGAQTWARVSRPPAPEAAGLFQGTFPDGFLWAVGSAAYQTEGGWQQHGKGASIWDTFTHHPLAPPGDSRNASLPLGAPSPLQPATGDVASDSYNNVFRDTEALRELGVTHYRFSISWARVLPNGSAGVPNREGLRYYRRLLERLRELGVQPVVTLYHWDLPQRLQDAYGGWANRALADHFRDYAELCFRHFGGQVKYWITIDNPYVVAWHGYATGRLAPGIRGSPRLGYLVAHNLLLAHAKVWHLYNTSFRPTQGGQVSIALSSHWINPRRMTDHSIKECQKSLDFVLGWFAKPVFIDGDYPESMKNNLSSILPDFTESEKKFIKGTADFFALCFGPTLSFQLLDPHMKFRQLESPNLRQLLSWIDLEFNHPQIFIVENGWFVSGTTKRDDAKYMYYLKKFIMETLKAIKLDGVDVIGYTAWSLMDGFEWHRGYSIRRGLFYVDFLSQDKMLLPKSSALFYQKLIEKNGFPPLPENQPLEGTFPCDFAWGVVDNYIQVSQLTKPISSLTKPYH

SEQ ID NO: 2 - protein, 550 aa, Mus musculus
MLARAPPRRPPRLVLLRLLLLHLLLLALRARCLSAEPGQGAQTWARFARAPAPEAAGLLHDTFPDGFLWAVGSAAYQTEGGWRQHGKGASIWDTFTHHSGAAPSDSPIVVAPSGAPSPPLSSTGDVASDSYNNVYRDTEGLRELGVTHYRFSISWARVLPNGTAGTPNREGLRYYRRLLERLRELGVQPVVTLYHWDLPQRLQDTYGGWANRALADHFRDYAELCFRHFGGQVKYWITIDNPYVVAWHGYATGRLAPGVRGSSRLGYLVAHNLLLAHAKVWHLYNTSFRPTQGGRVSIALSSHWINPRRMTDYNIRECQKSLDFVLGWFAKPIFIDGDYPESMKNNLSSLLPDFTESEKRLIRGTADFFALSFGPTLSFQLLDPNMKFRQLESPNLRQLLSWIDLEYNHPPIFIVENGWFVSGTTKRDDAKYMYYLKKFIMETLKAIRLDGVDVIGYTAWSLMDGFEWHRGYSIRRGLFYVDFLSQDKELLPKSSALFYQKLIEDNGFPPLPENQPLEGTFPCDFAWGVVDNYVQVSPLTKPSVGLLLPH

SEQ ID NO: 3 - DNA, 3024 bp, Artificial
  Gene construct comprising nucleotide sequence coding for Mus musculus klotho secreted splicing variant
tctagacatggctcgacagatctcaatattggccattagccatattattcattggttatatagcataaatcaatattggctattggccattgcatacgttgtatctatatcataatatgtacatttatattggctcatgtccaatatgaccgccatgttggcattgattattgactagttattaatagtaatcaattacggggtcattagttcatagcccatatatggagttccgcgttacataacttacggtaaatggcccgcctggctgaccgcccaacgacccccgcccattgacgtcaataatgacgtatgttcccatagtaacgccaatagggactttccattgacgtcaatgggtggagtatttacggtaaactgcccacttggcagtacatcaagtgtatcatatgccaagtccgccccctattgacgtcaatgacggtaaatggcccgcctggcattatgcccagtacatgaccttacgggactttcctacttggcagtacatctacgtattagtcatcgctattaccatggtgatgcggttttggcagtacaccaatgggcgtggatagcggtttgactcacggggatttccaagtctccaccccattgacgtcaatgggagtttgttttggcaccaaaatcaacgggactttccaaaatgtcgtaacaactgcgatcgcccgccccgttgacgcaaatgggcggtaggcgtgtacggtgggaggtctatataagcagagctcgtttagtgaaccgtcagatcactagaagctttattgcggtagtttatcacagttaaattgctaacgcagtcagtgcttctgacacaacagtctcgaacttaagctgcagtgactctcttaaggtagccttgcagaagttggtcgtgaggcactgggcaggtaagtatcaaggttacaagacaggtttaaggagaccaatagaaactgggcttgtcgagacagagaagactcttgcgtttctgataggcacctattggtcttactgacatccactttgcctttctctccacaggtgtccactcccagttcaattacagctcttaaggctagagtacttaatacgactcactataggctagcaatgctcgcccgcgcccctcctcgccgcccgccgcggctggtgctgctccgtttgctgttgctgcatctgctgctgctcgccctgcgcgcccgctgcctgagcgctgagccgggtcagggcgcgcagacctgggctcgcttcgcgcgcgctcctgccccagaggccgctggcctcctccacgacaccttccccgacggtttcctctgggcggtaggcagcgccgcctatcagaccgagggcggctggcgacagcacggcaaaggcgcgtccatctgggacactttcacccatcactctggggcggccccgtccgactccccgatcgtcgtggcgccgtcgggtgccccgtcgcctcccctgtcctccactggagatgtggccagcgatagttacaacaacgtctaccgcgacacagaggggctgcgcgaactgggggtcacccactaccgcttctccatatcgtgggcgcgggtgctccccaatggcaccgcgggcactcccaaccgcgaggggctgcgctactaccggcggctgctggagcggctgcgggagctgggcgtgcagccggtggttaccctgtaccattgggacctgccacagcgcctgcaggacacctatggcggatgggccaatcgcgccctggccgaccatttcagggattatgccgagctctgcttccgccacttcggtggtcaggtcaagtactggatcaccattgacaacccctacgtggtggcctggcacgggtatgccaccgggcgcctggccccgggcgtgaggggcagctccaggctcgggtacctggttgcccacaacctacttttggctcatgccaaagtctggcatctctacaacacctctttccgccccacacagggaggccgggtgtctatcgccttaagctcccattggatcaatcctcgaagaatgactgactataatatcagagaatgccagaagtctcttgactttgtgctaggctggtttgccaaacccatatttattgatggcgactacccagagagtatgaagaacaacctctcgtctcttctgcctgattttactgaatctgagaagaggctcatcagaggaactgctgacttttttgctctctccttcggaccaaccttgagctttcagctattggaccctaacatgaagttccgccaattggagtctcccaacctgaggcagcttctgtcttggatagatctggaatataaccaccctccaatatttattgtggaaaatggctggtttgtctcgggaaccaccaaaagggatgatgccaaatatatgtattatctcaagaagttcataatggaaaccttaaaagcaatcagactggatggggtcgacgtcattgggtacaccgcgtggtcgctcatggacggtttcgagtggcataggggctacagcatccggcgaggactcttctacgttgactttctgagtcaggacaaggagctgttgccaaagtcttcggccttgttctaccaaaagctgatagaggacaatggctttcctcctttacctgaaaaccagccccttgaagggacatttccctgtgactttgcttggggagttgttgacaactacgttcagctgagtcctttgacaaaacccagtgtcggcctcttgcttcctcactaagggccgcttccctttagtgagggttaatgcttcgagcagacatgataagatacattgatgagtttggacaaaccacaactagaatgcagtgaaaaaaatgctttatttgtgaaatttgtgatgctattgctttatttgtaaccattataagctgcaataaacaagttaacaacaacaattgcattcattttatgtttcaggttcagggggagatgtgggaggttttttaaagcaagtaaaacctctacaaatgtggta

SEQ ID NO: 4 - DNA, 3018 bp, Artificial
  Gene construct comprising nucleotide sequence coding for Homo sapiens klotho secreted splicing variant
tctagacatggctcgacagatctcaatattggccattagccatattattcattggttatatagcataaatcaatattggctattggccattgcatacgttgtatctatatcataatatgtacatttatattggctcatgtccaatatgaccgccatgttggcattgattattgactagttattaatagtaatcaattacggggtcattagttcatagcccatatatggagttccgcgttacataacttacggtaaatggcccgcctggctgaccgcccaacgacccccgcccattgacgtcaataatgacgtatgttcccatagtaacgccaatagggactttccattgacgtcaatgggtggagtatttacggtaaactgcccacttggcagtacatcaagtgtatcatatgccaagtccgccccctattgacgtcaatgacggtaaatggcccgcctggcattatgcccagtacatgaccttacgggactttcctacttggcagtacatctacgtattagtcatcgctattaccatggtgatgcggttttggcagtacaccaatgggcgtggatagcggtttgactcacggggatttccaagtctccaccccattgacgtcaatgggagtttgttttggcaccaaaatcaacgggactttccaaaatgtcgtaacaactgcgatcgcccgccccgttgacgcaaatgggcggtaggcgtgtacggtgggaggtctatataagcagagctcgtttagtgaaccgtcagatcactagaagctttattgcggtagtttatcacagttaaattgctaacgcagtcagtgcttctgacacaacagtctcgaacttaagctgcagtgactctcttaaggtagccttgcagaagttggtcgtgaggcactgggcaggtaagtatcaaggttacaagacaggtttaaggagaccaatagaaactgggcttgtcgagacagagaagactcttgcgtttctgataggcacctattggtcttactgacatccactttgcctttctctccacaggtgtccactcccagttcaattacagctcttaaggctagagtacttaatacgactcactataggctagcaatgcccgccagcgccccgccgcgccgcccgcggccgccgccgccgtcgctgtcgctgctgctggtgctgctgggcctgggcggccgccgcctgcgtgcggagccgggcgacggcgcgcagacctgggcccgtgtctcgcggcctcctgcccccgaggccgcgggcctcttccagggcaccttccccgacggcttcctctgggccgtgggcagcgccgcctaccagaccgagggcggctggcagcagcacggcaagggtgcgtccatctgggacacgttcacccaccaccccctggcacccccgggagactcccggaacgccagtctgccgttgggcgccccgtcgccgctgcagcccgccaccggggacgtagccagcgacagctacaacaacgtcttccgcgacacggaggcgctgcgcgagctcggggtcactcactaccgcttctccatctcgtgggcgcgagtgctccccaatggcagcgcgggcgtccccaaccgcgaggggctgcgctactaccggcgcctgctggagcggctgcgggagctgggcgtgcagcccgtggtcaccctgtaccactgggacctgccccagcgcctgcaggacgcctacggcggctgggccaaccgcgccctggccgaccacttcagggattacgcggagctctgcttccgccacttcggcggtcaggtcaagtactggatcaccatcgacaacccctacgtggtggcctggcacggctacgccaccgggcgcctggcccccggcatccggggcagcccgcggctcgggtacctggtggcgcacaacctcctcctggctcatgccaaagtctggcatctctacaatacttctttccgtcccactcagggaggtcaggtgtccattgccctaagctctcactggatcaatcctcgaagaatgaccgaccacagcatcaaagaatgtcaaaaatctctggactttgtactaggttggtttgccaaacccgtatttattgatggtgactatcccgagagcatgaagaataacctttcatctattctgcctgattttactgaatctgagaaaaagttcatcaaaggaactgctgacttttttgctctttgctttggacccaccttgagttttcaacttttggaccctcacatgaagttccgccaattggaatctcccaacctgaggcaactgctttcctggattgaccttgaatttaaccatcctcaaatatttattgtggaaaatggctggtttgtctcagggaccaccaagagagatgatgccaaatatatgtattacctcaaaaagttcatcatggaaaccttaaaagccatcaagctggatggggtggatgtcatcgggtataccgcatggtccctcatggatggtttcgagtggcacagaggttacagcatcaggcgtggactcttctatgttgactttctaagccaggacaagatgttgttgccaaagtcttcagccttgttctaccaaaagctgatagagaaaaatggcttccctcctttacctgaaaatcagcccctagaagggacatttccctgtgactttgcttggggagttgttgacaactacattcagctgagtcctttgacaaaacccagtgtcggcctcttgcttcctcactaagggccgcttccctttagtgagggttaatgcttcgagcagacatgataagatacattgatgagtttggacaaaccacaactagaatgcagtgaaaaaaatgctttatttgtgaaatttgtgatgctattgctttatttgtaaccattataagctgcaataaacaagttaacaacaacaattgcattcattttatgtttcaggttcagggggagatgtgggaggttttttaaagcaagtaaaacctctacaaatgtggta

SEQ ID NO: 5 - DNA, 1650 bp, Homo sapiens
atgcccgccagcgccccgccgcgccgcccgcggccgccgccgccgtcgctgtcgctgctgctggtgctgctgggcctgggcggccgccgcctgcgtgcggagccgggcgacggcgcgcagacctgggcccgtgtctcgcggcctcctgcccccgaggccgcgggcctcttccagggcaccttccccgacggcttcctctgggccgtgggcagcgccgcctaccagaccgagggcggctggcagcagcacggcaagggtgcgtccatctgggacacgttcacccaccaccccctggcacccccgggagactcccggaacgccagtctgccgttgggcgccccgtcgccgctgcagcccgccaccggggacgtagccagcgacagctacaacaacgtcttccgcgacacggaggcgctgcgcgagctcggggtcactcactaccgcttctccatctcgtgggcgcgagtgctccccaatggcagcgcgggcgtccccaaccgcgaggggctgcgctactaccggcgcctgctggagcggctgcgggagctgggcgtgcagcccgtggtcaccctgtaccactgggacctgccccagcgcctgcaggacgcctacggcggctgggccaaccgcgccctggccgaccacttcagggattacgcggagctctgcttccgccacttcggcggtcaggtcaagtactggatcaccatcgacaacccctacgtggtggcctggcacggctacgccaccgggcgcctggcccccggcatccggggcagcccgcggctcgggtacctggtggcgcacaacctcctcctggctcatgccaaagtctggcatctctacaatacttctttccgtcccactcagggaggtcaggtgtccattgccctaagctctcactggatcaatcctcgaagaatgaccgaccacagcatcaaagaatgtcaaaaatctctggactttgtactaggttggtttgccaaacccgtatttattgatggtgactatcccgagagcatgaagaataacctttcatctattctgcctgattttactgaatctgagaaaaagttcatcaaaggaactgctgacttttttgctctttgctttggacccaccttgagttttcaacttttggaccctcacatgaagttccgccaattggaatctcccaacctgaggcaactgctttcctggattgaccttgaatttaaccatcctcaaatatttattgtggaaaatggctggtttgtctcagggaccaccaagagagatgatgccaaatatatgtattacctcaaaaagttcatcatggaaaccttaaaagccatcaagctggatggggtggatgtcatcgggtataccgcatggtccctcatggatggtttcgagtggcacagaggttacagcatcaggcgtggactcttctatgttgactttctaagccaggacaagatgttgttgccaaagtcttcagccttgttctaccaaaagctgatagagaaaaatggcttccctcctttacctgaaaatcagcccctagaagggacatttccctgtgactttgcttggggagttgttgacaactacattcaagtaagtcagctgacaaaaccaatcagcagtctcaccaagccctatcactag

SEQ ID NO: 6 - DNA, 1653 bp, Mus musculus
atgctagcccgcgcccctcctcgccgcccgccgcggctggtgctgctccgtttgctgttgctgcatctgctgctgctcgccctgcgcgcccgctgcctgagcgctgagccgggtcagggcgcgcagacctgggctcgcttcgcgcgcgctcctgccccagaggccgctggcctcctccacgacaccttccccgacggtttcctctgggcggtaggcagcgccgcctatcagaccgagggcggctggcgacagcacggcaaaggcgcgtccatctgggacactttcacccatcactctggggcggccccgtccgactccccgatcgtcgtggcgccgtcgggtgccccgtcgcctcccctgtcctccactggagatgtggccagcgatagttacaacaacgtctaccgcgacacagaggggctgcgcgaactgggggtcacccactaccgcttctccatatcgtgggcgcgggtgctccccaatggcaccgcgggcactcccaaccgcgaggggctgcgctactaccggcggctgctggagcggctgcgggagctgggcgtgcagccggtggttaccctgtaccattgggacctgccacagcgcctgcaggacacctatggcggatgggccaatcgcgccctggccgaccatttcagggattatgccgagctctgcttccgccacttcggtggtcaggtcaagtactggatcaccattgacaacccctacgtggtggcctggcacgggtatgccaccgggcgcctggccccgggcgtgaggggcagctccaggctcgggtacctggttgcccacaacctacttttggctcatgccaaagtctggcatctctacaacacctctttccgccccacacagggaggccgggtgtctatcgccttaagctcccattggatcaatcctcgaagaatgactgactataatatcagagaatgccagaagtctcttgactttgtgctaggctggtttgccaaacccatatttattgatggcgactacccagagagtatgaagaacaacctctcgtctcttctgcctgattttactgaatctgagaagaggctcatcagaggaactgctgacttttttgctctctccttcggaccaaccttgagctttcagctattggaccctaacatgaagttccgccaattggagtctcccaacctgaggcagcttctgtcttggatagatctggaatataaccaccctccaatatttattgtggaaaatggctggtttgtctcgggaaccaccaaaagggatgatgccaaatatatgtattatctcaagaagttcataatggaaaccttaaaagcaatcagactggatggggtcgacgtcattgggtacaccgcgtggtcgctcatggacggtttcgagtggcataggggctacagcatccggcgaggactcttctacgttgactttctgagtcaggacaaggagctgttgccaaagtcttcggccttgttctaccaaaagctgatagaggacaatggctttcctcctttacctgaaaaccagccccttgaagggacatttccctgtgactttgcttggggagttgttgacaactacgttcaagtaagtcctttgacaaaacccagtgtcggcctcttgcttcctcactaa

SEQ ID NO: 7 - DNA, 20 bp, Artificial
  forward primer
ttcaaacccggaagtctttg

SEQ ID NO: 8 - DNA, 20 bp, Artificial
  Reverse primer
ccaggcagacgttcacatta

SEQ ID NO: 9 - DNA, 20 bp, Artificial
  Forward primer
tggctttcctcctttacctg

SEQ ID NO: 10 - DNA, 18 bp, Artificial
  Reverse primer
gccgacactgggttttgt

SEQ ID NO: 11 - protein, 14 aa, Mus musculus
SPLTKPSVGLLLPH

SEQ ID NO: 12 - DNA, 5421 bp, Artificial
  Plasmid pGG2
  promoter (206)..(955): CMV IE enhancer/promoter
  Intron (1095)..(1227): Intron from pCl-neo
  misc_feature (1227)..(1334): Multiple Cloning Site (MCS)
  polyA_signal (1369)..(1590): SV40 late poly A signal
cagcagctgcgcgctcgctcgctcactgaggccgcccgggcaaagcccgggcgtcgggcgacctttggtcgcccggcctcagtgagcgagcgagcgcgcagagagggagtggccaactccatcactaggggttccttgtagttaatgattaacccgccatgctacttatctacgtagccatgctctagacatggctcgacagatctcaatattggccattagccatattattcattggttatatagcataaatcaatattggctattggccattgcatacgttgtatctatatcataatatgtacatttatattggctcatgtccaatatgaccgccatgttggcattgattattgactagttattaatagtaatcaattacggggtcattagttcatagcccatatatggagttccgcgttacataacttacggtaaatggcccgcctggctgaccgcccaacgacccccgcccattgacgtcaataatgacgtatgttcccatagtaacgccaatagggactttccattgacgtcaatgggtggagtatttacggtaaactgcccacttggcagtacatcaagtgtatcatatgccaagtccgccccctattgacgtcaatgacggtaaatggcccgcctggcattatgcccagtacatgaccttacgggactttcctacttggcagtacatctacgtattagtcatcgctattaccatggtgatgcggttttggcagtacaccaatgggcgtggatagcggtttgactcacggggatttccaagtctccaccccattgacgtcaatgggagtttgttttggcaccaaaatcaacgggactttccaaaatgtcgtaacaactgcgatcgcccgccccgttgacgcaaatgggcggtaggcgtgtacggtgggaggtctatataagcagagctcgtttagtgaaccgtcagatcactagaagctttattgcggtagtttatcacagttaaattgctaacgcagtcagtgcttctgacacaacagtctcgaacttaagctgcagtgactctcttaaggtagccttgcagaagttggtcgtgaggcactgggcaggtaagtatcaaggttacaagacaggtttaaggagaccaatagaaactgggcttgtcgagacagagaagactcttgcgtttctgataggcacctattggtcttactgacatccactttgcctttctctccacaggtgtccactcccagttcaattacagctcttaaggctagagtacttaatacgactcactataggctagcctcgacctcgagacgcgtgatatcggatcccggccggcggccgcttccctttagtgagggttaatgcttcgagcagacatgataagatacattgatgagtttggacaaaccacaactagaatgcagtgaaaaaaatgctttatttgtgaaatttgtgatgctattgctttatttgtaaccattataagctgcaataaacaagttaacaacaacaattgcattcattttatgtttcaggttcagggggagatgtgggaggttttttaaagcaagtaaaacctctacaaatgtggtaaaatccgataagggactagagcatggctacgtagataagtagcatggcgggttaatcattaactacaaggaacccctagtgatggagttggccactccctctctgcgcgctcgctcgctcactgaggccgggcgaccaaaggtcgcccgacgcccgggctttgcccgggcggcctcagtgagcgagcgagcgcgccagctggcgtaatagcgaagaggcccgcaccgatcgcccttcccaacagttgcgcagcctgaatggcgaatggaattccagacgattgagcgtcaaaatgtaggtatttccatgagcgtttttccgttgcaatggctggcggtaatattgttctggatattaccagcaaggccgatagtttgagttcttctactcaggcaagtgatgttattactaatcaaagaagtattgcgacaacggttaatttgcgtgatggacagactcttttactcggtggcctcactgattataaaaacacttctcaggattctggcgtaccgttcctgtctaaaatccctttaatcggcctcctgtttagctcccgctctgattctaacgaggaaagcacgttatacgtgctcgtcaaagcaaccatagtacgcgccctgtagcggcgcattaagcgcggcgggtgtggtggttacgcgcagcgtgaccgctacacttgccagcgccctagcgcccgctcctttcgctttcttcccttcctttctcgccacgttcgccggctttccccgtcaagctctaaatcgggggctccctttagggttccgatttagtgctttacggcacctcgaccccaaaaaacttgattagggtgatggttcacgtagtgggccatcgccctgatagacggtttttcgccctttgacgttggagtccacgttctttaatagtggactcttgttccaaactggaacaacactcaaccctatctcggtctattcttttgatttataagggattttgccgatttcggcctattggttaaaaaatgagctgatttaacaaaaatttaacgcgaattttaacaaaatattaacgtctacaatttaaatatttgcttatacaatcttcctgtttttggggcttttctgattatcaaccggggtacatatgattgacatgctagttttacgattaccgttcatcgattctcttgtttgctccagactctcaggcaatgacctgatagcctttgtagagacctctcaaaaatagctaccctctccggcatgaatttatcagctagaacggttgaatatcatattgatggtgatttgactgtctccggcctttctcacccgtttgaatctttacctacacattactcaggcattgcatttaaaatatatgagggttctaaaaatttttatccttgcgttgaaataaaggcttctcccgcaaaagtattacagggtcataatgtttttggtacaaccgatttagctttatgctctgaggctttattgcttaattttgctaattctttgccttgcctgtatgatttattggatgttggaatcgcctgatgcggtattttctccttacgcatctgtgcggtatttcacaccgcatatggtgcactctcagtacaatctgctctgatgccgcatagttaagccagccccgacacccgccaacacccgctgacgcgccctgacgggcttgtctgctcccggcatccgcttacagacaagctgtgaccgtctccgggagctgcatgtgtcagaggttttcaccgtcatcaccgaaacgcgcgagacgaaagggcctcgtgatacgcctatttttataggttaatgtcatgataataatggtttcttagacgtcaggtggcacttttcggggaaatgtgcgcggaacccctatttgtttatttttctaaatacattcaaatatgtatccgctcatgagacaataaccctgataaatgcttcaataatattgaaaaaggaagagtatgagtattcaacatttccgtgtcgcccttattcccttttttgcggcattttgccttcctgtttttgctcacccagaaacgctggtgaaagtaaaagatgctgaagatcagttgggtgcacgagtgggttacatcgaactggatctcaacagcggtaagatccttgagagttttcgccccgaagaacgttttccaatgatgagcacttttaaagttctgctatgtggcgcggtattatcccgtattgacgccgggcaagagcaactcggtcgccgcatacactattctcagaatgacttggttgagtactcaccagtcacagaaaagcatcttacggatggcatgacagtaagagaattatgcagtgctgccataaccatgagtgataacactgcggccaacttacttctgacaacgatcggaggaccgaaggagctaaccgcttttttgcacaacatgggggatcatgtaactcgccttgatcgttgggaaccggagctgaatgaagccataccaaacgacgagcgtgacaccacgatgcctgtagcaatggcaacaacgttgcgcaaactattaactggcgaactacttactctagcttcccggcaacaattaatagactggatggaggcggataaagttgcaggaccacttctgcgctcggcccttccggctggctggtttattgctgataaatctggagccggtgagcgtgggtctcgcggtatcattgcagcactggggccagatggtaagccctcccgtatcgtagttatctacacgacggggagtcaggcaactatggatgaacgaaatagacagatcgctgagataggtgcctcactgattaagcattggtaactgtcagaccaagtttactcatatatactttagattgatttaaaacttcatttttaatttaaaaggatctaggtgaagatcctttttgataatctcatgaccaaaatcccttaacgtgagttttcgttccactgagcgtcagaccccgtagaaaagatcaaaggatcttcttgagatcctttttttctgcgcgtaatctgctgcttgcaaacaaaaaaaccaccgctaccagcggtggtttgtttgccggatcaagagctaccaactctttttccgaaggtaactggcttcagcagagcgcagataccaaatactgtccttctagtgtagccgtagttaggccaccacttcaagaactctgtagcaccgcctacatacctcgctctgctaatcctgttaccagtggctgctgccagtggcgataagtcgtgtcttaccgggttggactcaagacgatagttaccggataaggcgcagcggtcgggctgaacggggggttcgtgcacacagcccagcttggagcgaacgacctacaccgaactgagatacctacagcgtgagctatgagaaagcgccacgcttcccgaagggagaaaggcggacaggtatccggtaagcggcagggtcggaacaggagagcgcacgagggagcttccagggggaaacgcctggtatctttatagtcctgtcgggtttcgccacctctgacttgagcgtcgatttttgtgatgctcgtcaggggggcggagcctatggaaaaacgccagcaacgcggcctttttacggttcctggccttttgctggccttttgctcacatgttctttcctgcgttatcccctgattctgtggataaccgtattaccgcctttgagtgagctgataccgctcgccgcagccgaacgaccgagcgcagcgagtcagtgagcgaggaagcggaagagcgcccaatacgcaaaccgcctctccccgcgcgttggccgattcattaatg

SEQ ID NO: 13 - DNA, 8335 bp, Artificial
  pGG2 plasmid comprising sequences of CMV IE promoter and the sequence coding for mouse m-KL (pGG2-m-KL)
cagcagctgcgcgctcgctcgctcactgaggccgcccgggcaaagcccgggcgtcgggcgacctttggtcgcccggcctcagtgagcgagcgagcgcgcagagagggagtggccaactccatcactaggggttccttgtagttaatgattaacccgccatgctacttatctacgtagccatgctctagacatggctcgacagatctcaatattggccattagccatattattcattggttatatagcataaatcaatattggctattggccattgcatacgttgtatctatatcataatatgtacatttatattggctcatgtccaatatgaccgccatgttggcattgattattgactagttattaatagtaatcaattacggggtcattagttcatagcccatatatggagttccgcgttacataacttacggtaaatggcccgcctggctgaccgcccaacgacccccgcccattgacgtcaataatgacgtatgttcccatagtaacgccaatagggactttccattgacgtcaatgggtggagtatttacggtaaactgcccacttggcagtacatcaagtgtatcatatgccaagtccgccccctattgacgtcaatgacggtaaatggcccgcctggcattatgcccagtacatgaccttacgggactttcctacttggcagtacatctacgtattagtcatcgctattaccatggtgatgcggttttggcagtacaccaatgggcgtggatagcggtttgactcacggggatttccaagtctccaccccattgacgtcaatgggagtttgttttggcaccaaaatcaacgggactttccaaaatgtcgtaacaactgcgatcgcccgccccgttgacgcaaatgggcggtaggcgtgtacggtgggaggtctatataagcagagctcgtttagtgaaccgtcagatcactagaagcttgatatcgaattcgcccttgataatcattgctcgtggggcggcgggagcgggggtgggcaccgcgtagggagggcggcggggcgcgggcatataggggcgcggcgcggtgccctcccggctcccgcagcatgctagcccgcgcccctcctcgccgcccgccgcggctggtgctgctccgtttgctgttgctgcatctgctgctgctcgccctgcgcgcccgctgcctgagcgctgagccgggtcagggcgcgcagacctgggctcgcttcgcgcgcgctcctgccccagaggccgctggcctcctccacgacaccttccccgacggtttcctctgggcggtaggcagcgccgcctatcagaccgagggcggctggcgacagcacggcaaaggcgcgtccatctgggacactttcacccatcactctggggcggccccgtccgactccccgatcgtcgtggcgccgtcgggtgccccgtcgcctcccctgtcctccactggagatgtggccagcgatagttacaacaacgtctaccgcgacacagaggggctgcgcgaactgggggtcacccactaccgcttctccatatcgtgggcgcgggtgctccccaatggcaccgcgggcactcccaaccgcgaggggctgcgctactaccggcggctgctggagcggctgcgggagctgggcgtgcagccggtggttaccctgtaccattgggacctgccacagcgcctgcaggacacctatggcggatgggccaatcgcgccctggccgaccatttcagggattatgccgagctctgcttccgccacttcggtggtcaggtcaagtactggatcaccattgacaacccctacgtggtggcctggcacgggtatgccaccgggcgcctggccccgggcgtgaggggcagctccaggctcgggtacctggttgcccacaacctacttttggctcatgccaaagtctggcatctctacaacacctctttccgccccacacagggaggccgggtgtctatcgccttaagctcccattggatcaatcctcgaagaatgactgactataatatcagagaatgccagaagtctcttgactttgtgctaggctggtttgccaaacccatatttattgatggcgactacccagagagtatgaagaacaacctctcgtctcttctgcctgattttactgaatctgagaagaggctcatcagaggaactgctgacttttttgctctctccttcggaccaaccttgagctttcagctattggaccctaacatgaagttccgccaattggagtctcccaacctgaggcagcttctgtcttggatagatctggaatataaccaccctccaatatttattgtggaaaatggctggtttgtctcgggaaccaccaaaagggatgatgccaaatatatgtattatctcaagaagttcataatggaaaccttaaaagcaatcagactggatggggtcgacgtcattgggtacaccgcgtggtcgctcatggacggtttcgagtggcataggggctacagcatccggcgaggactcttctacgttgactttctgagtcaggacaaggagctgttgccaaagtcttcggccttgttctaccaaaagctgatagaggacaatggctttcctcctttacctgaaaaccagccccttgaagggacatttccctgtgactttgcttggggagttgttgacaactacgttcaagtggacactactctctctcagtttactgacccgaatgtctatctgtgggatgtgcatcacagtaagaggcttattaaagtagacggggttgtagccaagaagagaaaaccttactgtgttgatttctctgccatccggcctcagataaccttacttcgagaaatgcgggtcacccactttcgcttctccctggactgggccctgatcttgcctctgggtaaccagacccaagtgaaccacacggttctgcacttctaccgctgcatgatcagcgagctggtgcacgccaacatcactccagtggtggccctgtggcagccagcagccccgcaccaaggcctgccacatgcccttgcaaaacatggggcctgggagaacccgcacactgctctggcgtttgcagactacgcaaacctgtgttttaaagagttgggtcactgggtcaatctctggatcaccatgaacgagccaaacacacggaacatgacctatcgtgccgggcaccacctcctgagagcccatgccttggcttggcatctgtacgatgacaagtttagggcggctcagaaaggcaaaatatccatcgccttgcaggctgactggatagaaccggcctgccctttctctcaaaatgacaaagaagtggccgagagagttttggaatttgatataggctggctggcagagcctatttttggttccggagattatccacgtgtgatgagggactggctgaaccaaaaaaacaattttcttttgccctatttcaccgaagatgaaaaaaagctagtccggggttcctttgacttcctggcggtgagtcattacaccaccattctggtagactgggaaaaggaggatccgatgaaatacaacgattacttggaggtacaggagatgactgacatcacatggctcaactctcccagtcaggtggcagtggtgccttgggggctgcgcaaagtgctcaactggctaaggttcaagtacggagacctcccgatgtatgtgacagccaatggaatcgatgatgacccccacgccgagcaagactcactgaggatctattatattaagaattatgtgaatgaggctctgaaagcctacgtgttggacgacatcaacctttgtggctactttgcgtattcacttagtgatcgctcagctcccaagtctggcttttatcgatatgctgcgaatcagtttgagcccaaaccatctatgaaacattacaggaaaattattgacagcaatggcttcctgggttctggaacactgggaaggttttgtccagaagaatacactgtgtgcaccgaatgtggattttttcaaacccggaagtctttgctggtcttcatctcgtttcttgtttttacttttattatttctcttgctctcatttttcactactccaagaaaggccagagaagttataagtaatgtgaacgtctgcctggccattcgctttgggatcaagatgtacacgccgtcagccgtttgcacctctctgtgttgtgagccgcattccacacatttcgattctagagcggccgcttccctttagtgagggttaatgcttcgagcagacatgataagatacattgatgagtttggacaaaccacaactagaatgcagtgaaaaaaatgctttatttgtgaaatttgtgatgctattgctttatttgtaaccattataagctgcaataaacaagttaacaacaacaattgcattcattttatgtttcaggttcagggggagatgtgggaggttttttaaagcaagtaaaacctctacaaatgtggtaaaatccgataagggactagagcatggctacgtagataagtagcatggcgggttaatcattaactacaaggaacccctagtgatggagttggccactccctctctgcgcgctcgctcgctcactgaggccgggcgaccaaaggtcgcccgacgcccgggctttgcccgggcggcctcagtgagcgagcgagcgcgccagctggcgtaatagcgaagaggcccgcaccgatcgcccttcccaacagttgcgcagcctgaatggcgaatggaattccagacgattgagcgtcaaaatgtaggtatttccatgagcgtttttccgttgcaatggctggcggtaatattgttctggatattaccagcaaggccgatagtttgagttcttctactcaggcaagtgatgttattactaatcaaagaagtattgcgacaacggttaatttgcgtgatggacagactcttttactcggtggcctcactgattataaaaacacttctcaggattctggcgtaccgttcctgtctaaaatccctttaatcggcctcctgtttagctcccgctctgattctaacgaggaaagcacgttatacgtgctcgtcaaagcaaccatagtacgcgccctgtagcggcgcattaagcgcggcgggtgtggtggttacgcgcagcgtgaccgctacacttgccagcgccctagcgcccgctcctttcgctttcttcccttcctttctcgccacgttcgccggctttccccgtcaagctctaaatcgggggctccctttagggttccgatttagtgctttacggcacctcgaccccaaaaaacttgattagggtgatggttcacgtagtgggccatcgccctgatagacggtttttcgccctttgacgttggagtccacgttctttaatagtggactcttgttccaaactggaacaacactcaaccctatctcggtctattcttttgatttataagggattttgccgatttcggcctattggttaaaaaatgagctgatttaacaaaaatttaacgcgaattttaacaaaatattaacgtctacaatttaaatatttgcttatacaatcttcctgtttttggggcttttctgattatcaaccggggtacatatgattgacatgctagttttacgattaccgttcatcgattctcttgtttgctccagactctcaggcaatgacctgatagcctttgtagagacctctcaaaaatagctaccctctccggcatgaatttatcagctagaacggttgaatatcatattgatggtgatttgactgtctccggcctttctcacccgtttgaatctttacctacacattactcaggcattgcatttaaaatatatgagggttctaaaaatttttatccttgcgttgaaataaaggcttctcccgcaaaagtattacagggtcataatgtttttggtacaaccgatttagctttatgctctgaggctttattgcttaattttgctaattctttgccttgcctgtatgatttattggatgttggaatcgcctgatgcggtattttctccttacgcatctgtgcggtatttcacaccgcatatggtgcactctcagtacaatctgctctgatgccgcatagttaagccagccccgacacccgccaacacccgctgacgcgccctgacgggcttgtctgctcccggcatccgcttacagacaagctgtgaccgtctccgggagctgcatgtgtcagaggttttcaccgtcatcaccgaaacgcgcgagacgaaagggcctcgtgatacgcctatttttataggttaatgtcatgataataatggtttcttagacgtcaggtggcacttttcggggaaatgtgcgcggaacccctatttgtttatttttctaaatacattcaaatatgtatccgctcatgagacaataaccctgataaatgcttcaataatattgaaaaaggaagagtatgagtattcaacatttccgtgtcgcccttattcccttttttgcggcattttgccttcctgtttttgctcacccagaaacgctggtgaaagtaaaagatgctgaagatcagttgggtgcacgagtgggttacatcgaactggatctcaacagcggtaagatccttgagagttttcgccccgaagaacgttttccaatgatgagcacttttaaagttctgctatgtggcgcggtattatcccgtattgacgccgggcaagagcaactcggtcgccgcatacactattctcagaatgacttggttgagtactcaccagtcacagaaaagcatcttacggatggcatgacagtaagagaattatgcagtgctgccataaccatgagtgataacactgcggccaacttacttctgacaacgatcggaggaccgaaggagctaaccgcttttttgcacaacatgggggatcatgtaactcgccttgatcgttgggaaccggagctgaatgaagccataccaaacgacgagcgtgacaccacgatgcctgtagcaatggcaacaacgttgcgcaaactattaactggcgaactacttactctagcttcccggcaacaattaatagactggatggaggcggataaagttgcaggaccacttctgcgctcggcccttccggctggctggtttattgctgataaatctggagccggtgagcgtgggtctcgcggtatcattgcagcactggggccagatggtaagccctcccgtatcgtagttatctacacgacggggagtcaggcaactatggatgaacgaaatagacagatcgctgagataggtgcctcactgattaagcattggtaactgtcagaccaagtttactcatatatactttagattgatttaaaacttcatttttaatttaaaaggatctaggtgaagatcctttttgataatctcatgaccaaaatcccttaacgtgagttttcgttccactgagcgtcagaccccgtagaaaagatcaaaggatcttcttgagatcctttttttctgcgcgtaatctgctgcttgcaaacaaaaaaaccaccgctaccagcggtggtttgtttgccggatcaagagctaccaactctttttccgaaggtaactggcttcagcagagcgcagataccaaatactgtccttctagtgtagccgtagttaggccaccacttcaagaactctgtagcaccgcctacatacctcgctctgctaatcctgttaccagtggctgctgccagtggcgataagtcgtgtcttaccgggttggactcaagacgatagttaccggataaggcgcagcggtcgggctgaacggggggttcgtgcacacagcccagcttggagcgaacgacctacaccgaactgagatacctacagcgtgagctatgagaaagcgccacgcttcccgaagggagaaaggcggacaggtatccggtaagcggcagggtcggaacaggagagcgcacgagggagcttccagggggaaacgcctggtatctttatagtcctgtcgggtttcgccacctctgacttgagcgtcgatttttgtgatgctcgtcaggggggcggagcctatggaaaaacgccagcaacgcggcctttttacggttcctggccttttgctggccttttgctcacatgttctttcctgcgttatcccctgattctgtggataaccgtattaccgcctttgagtgagctgataccgctcgccgcagccgaacgaccgagcgcagcgagtcagtgagcgaggaagcggaagagcgcccaatacgcaaaccgcctctccccgcgcgttggccgattcattaatg

SEQ ID NO: 14 - DNA, 5640 bp, Artificial
  synthetic plasmid pUC57-KL (GenScript, USA)
tcgcgcgtttcggtgatgacggtgaaaacctctgacacatgcagctcccggagacggtcacagcttgtctgtaagcggatgccgggagcagacaagcccgtcagggcgcgtcagcgggtgttggcgggtgtcggggctggcttaactatgcggcatcagagcagattgtactgagagtgcaccatatgcggtgtgaaataccgcacagatgcgtaaggagaaaataccgcatcaggcgccattcgccattcaggctgcgcaactgttgggaagggcgatcggtgcgggcctcttcgctattacgccagctggcgaaagggggatgtgctgcaaggcgattaagttgggtaacgccagggttttcccagtcacgacgttgtaaaacgacggccagtgaattcttctagaatgctcgcccgcgcccctcctcgccgcccgccgcggctggtgctgctccgtttgctgttgctgcatctgctgctgctcgccctgcgcgcccgctgcctgagcgctgagccgggtcagggcgcgcagacctgggctcgcttcgcgcgcgctcctgccccagaggccgctggcctcctccacgacaccttccccgacggtttcctctgggcggtaggcagcgccgcctatcagaccgagggcggctggcgacagcacggcaaaggcgcgtccatctgggacactttcacccatcactctggggcggccccgtccgactccccgatcgtcgtggcgccgtcgggtgccccgtcgcctcccctgtcctccactggagatgtggccagcgatagttacaacaacgtctaccgcgacacagaggggctgcgcgaactgggggtcacccactaccgcttctccatatcgtgggcgcgggtgctccccaatggcaccgcgggcactcccaaccgcgaggggctgcgctactaccggcggctgctggagcggctgcgggagctgggcgtgcagccggtggttaccctgtaccattgggacctgccacagcgcctgcaggacacctatggcggatgggccaatcgcgccctggccgaccatttcagggattatgccgagctctgcttccgccacttcggtggtcaggtcaagtactggatcaccattgacaacccctacgtggtggcctggcacgggtatgccaccgggcgcctggccccgggcgtgaggggcagctccaggctcgggtacctggttgcccacaacctacttttggctcatgccaaagtctggcatctctacaacacctctttccgccccacacagggaggccgggtgtctatcgccttaagctcccattggatcaatcctcgaagaatgactgactataatatcagagaatgccagaagtctcttgactttgtgctaggctggtttgccaaacccatatttattgatggcgactacccagagagtatgaagaacaacctctcgtctcttctgcctgattttactgaatctgagaagaggctcatcagaggaactgctgacttttttgctctctccttcggaccaaccttgagctttcagctattggaccctaacatgaagttccgccaattggagtctcccaacctgaggcagcttctgtcttggatagatctggaatataaccaccctccaatatttattgtggaaaatggctggtttgtctcgggaaccaccaaaagggatgatgccaaatatatgtattatctcaagaagttcataatggaaaccttaaaagcaatcagactggatggggtcgacgtcattgggtacaccgcgtggtcgctcatggacggtttcgagtggcataggggctacagcatccggcgaggactcttctacgttgactttctgagtcaggacaaggagctgttgccaaagtcttcggccttgttctaccaaaagctgatagaggacaatggctttcctcctttacctgaaaaccagccccttgaagggacatttccctgtgactttgcttggggagttgttgacaactacgttcagctgagtcctttgacaaaacccagtgtcggcctcttgcttcctcactaagggcccagagactgaagctttacgtagacactactctctctcagtttactgacccgaatgtctatctgtgggatgtgcatcacagtaagaggcttattaaagtagacggggttgtagccaaggctagcaaaccttactgtgttgatttctctgccatccggcctcagataaccttacttcgagaaatgcgggtcacccactttcgcttctccctggactgggcgctgatcttgcctctgggtaaccagacccaagtgaaccacacggttctgcacttctaccgctgcatgatcagcgagctggtgcacgccaacatcactccagtggtggccctgtggcagccagcagccccgcaccaaggcctgccacatgcccttgcaaaacatggggcctgggagaacccgcacactgctctggcgtttgcagactacgcaaacctgtgttttaaagagttgggtcactgggtcaatctctggatcaccatgaacgagccaaacacacggaacatgacctatcgtgccgggcaccacctcctgagagcccatgccttggcttggcatctgtacgatgacaagtttagggcggctcagaaaggcaaaatatccatcgccttgcaggctgactggatagaaccggcctgccctttctctcaaaatgacaaagaagtggccgagagagttttggaatttgatataggctggctggcagagcctatttttggttccggagattatccacgtgtgatgagggactggctgaaccaaaaaaacaattttcttttgccctatttcaccgaagatgaaaaaaagctagtccggggttcctttgacttcctggcggtgagtcattacaccaccattctggtagactgggaaaaggaggatccgatgaaatacaacgattacttggaggtacaggagatgactgacatcacatggctcaactctcccagtcaggtggcagtggtgccttgggggctgcgcaaagtgctcaactggctaaggttcaagtacggagacctcccgatgtatgtgacagccaatggaatcgatgatgacccccacgccgagcaagactcactgaggatctattatattaagaattatgtgaatgaggctctgaaagcctacgtgttggacgacatcaacctttgtggctactttgcgtattcacttagtgatcgctcagctcccaagtctggcttttatcgatatgctgcgaatcagtttgagcccaaaccatctatgaaacattacaggaaaattattgacagcaatggcttcctgggttctggaacactgggaaggttttgtccagaagaataagcggccgcgcatgcaagcttggcgtaatcatggtcatagctgtttcctgtgtgaaattgttatccgctcacaattccacacaacatacgagccggaagcataaagtgtaaagcctggggtgcctaatgagtgagctaactcacattaattgcgttgcgctcactgcccgctttccagtcgggaaacctgtcgtgccagctgcattaatgaatcggccaacgcgcggggagaggcggtttgcgtattgggcgctcttccgcttcctcgctcactgactcgctgcgctcggtcgttcggctgcggcgagcggtatcagctcactcaaaggcggtaatacggttatccacagaatcaggggataacgcaggaaagaacatgtgagcaaaaggccagcaaaaggccaggaaccgtaaaaaggccgcgttgctggcgtttttccataggctccgcccccctgacgagcatcacaaaaatcgacgctcaagtcagaggtggcgaaacccgacaggactataaagataccaggcgtttccccctggaagctccctcgtgcgctctcctgttccgaccctgccgcttaccggatacctgtccgcctttctcccttcgggaagcgtggcgctttctcatagctcacgctgtaggtatctcagttcggtgtaggtcgttcgctccaagctgggctgtgtgcacgaaccccccgttcagcccgaccgctgcgccttatccggtaactatcgtcttgagtccaacccggtaagacacgacttatcgccactggcagcagccactggtaacaggattagcagagcgaggtatgtaggcggtgctacagagttcttgaagtggtggcctaactacggctacactagaagaacagtatttggtatctgcgctctgctgaagccagttaccttcggaaaaagagttggtagctcttgatccggcaaacaaaccaccgctggtagcggtggtttttttgtttgcaagcagcagattacgcgcagaaaaaaaggatctcaagaagatcctttgatcttttctacggggtctgacgctcagtggaacgaaaactcacgttaagggattttggtcatgagattatcaaaaaggatcttcacctagatccttttaaattaaaaatgaagttttaaatcaatctaaagtatatatgagtaaacttggtctgacagttaccaatgcttaatcagtgaggcacctatctcagcgatctgtctatttcgttcatccatagttgcctgactccccgtcgtgtagataactacgatacgggagggcttaccatctggccccagtgctgcaatgataccgcgagacccacgctcaccggctccagatttatcagcaataaaccagccagccggaagggccgagcgcagaagtggtcctgcaactttatccgcctccatccagtctattaattgttgccgggaagctagagtaagtagttcgccagttaatagtttgcgcaacgttgttgccattgctacaggcatcgtggtgtcacgctcgtcgtttggtatggcttcattcagctccggttcccaacgatcaaggcgagttacatgatcccccatgttgtgcaaaaaagcggttagctccttcggtcctccgatcgttgtcagaagtaagttggccgcagtgttatcactcatggttatggcagcactgcataattctcttactgtcatgccatccgtaagatgcttttctgtgactggtgagtactcaaccaagtcattctgagaatagtgtatgcggcgaccgagttgctcttgcccggcgtcaatacgggataataccgcgccacatagcagaactttaaaagtgctcatcattggaaaacgttcttcggggcgaaaactctcaaggatcttaccgctgttgagatccagttcgatgtaacccactcgtgcacccaactgatcttcagcatcttttactttcaccagcgtttctgggtgagcaaaaacaggaaggcaaaatgccgcaaaaaagggaataagggcgacacggaaatgttgaatactcatactcttcctttttcaatattattgaagcatttatcagggttattgtctcatgagcggatacatatttgaatgtatttagaaaaataaacaaataggggttccgcgcacatttccccgaaaagtgccacctgacgtctaagaaaccattattatcatgacattaacctataaaaataggcgtatcacgaggccctttcgtc

SEQ ID NO: 15 - DNA, 5931 bp, Artificial
  pGG2 plasmid comprising sequences of CMV IE promoter and the sequence coding for mouse s-KL (pGG2-s-KL)
cagcagctgcgcgctcgctcgctcactgaggccgcccgggcaaagcccgggcgtcgggcgacctttggtcgcccggcctcagtgagcgagcgagcgcgcagagagggagtggccaactccatcactaggggttccttgtagttaatgattaacccgccatgctacttatctacgtagccatgctctagaatgctcgcccgcgcccctcctcgccgcccgccgcggctggtgctgctccgtttgctgttgctgcatctgctgctgctcgccctgcgcgcccgctgcctgagcgctgagccgggtcagggcgcgcagacctgggctcgcttcgcgcgcgctcctgccccagaggccgctggcctcctccacgacaccttccccgacggtttcctctgggcggtaggcagcgccgcctatcagaccgagggcggctggcgacagcacggcaaaggcgcgtccatctgggacactttcacccatcactctggggcggccccgtccgactccccgatcgtcgtggcgccgtcgggtgccccgtcgcctcccctgtcctccactggagatgtggccagcgatagttacaacaacgtctaccgcgacacagaggggctgcgcgaactgggggtcacccactaccgcttctccatatcgtgggcgcgggtgctccccaatggcaccgcgggcactcccaaccgcgaggggctgcgctactaccggcggctgctggagcggctgcgggagctgggcgtgcagccggtggttaccctgtaccattgggacctgccacagcgcctgcaggacacctatggcggatgggccaatcgcgccctggccgaccatttcagggattatgccgagctctgcttccgccacttcggtggtcaggtcaagtactggatcaccattgacaacccctacgtggtggcctggcacgggtatgccaccgggcgcctggccccgggcgtgaggggcagctccaggctcgggtacctggttgcccacaacctacttttggctcatgccaaagtctggcatctctacaacacctctttccgccccacacagggaggccgggtgtctatcgccttaagctcccattggatcaatcctcgaagaatgactgactataatatcagagaatgccagaagtctcttgactttgtgctaggctggtttgccaaacccatatttattgatggcgactacccagagagtatgaagaacaacctctcgtctcttctgcctgattttactgaatctgagaagaggctcatcagaggaactgctgacttttttgctctctccttcggaccaaccttgagctttcagctattggaccctaacatgaagttccgccaattggagtctcccaacctgaggcagcttctgtcttggatagatctggaatataaccaccctccaatatttattgtggaaaatggctggtttgtctcgggaaccaccaaaagggatgatgccaaatatatgtattatctcaagaagttcataatggaaaccttaaaagcaatcagactggatggggtcgacgtcattgggtacaccgcgtggtcgctcatggacggtttcgagtggcataggggctacagcatccggcgaggactcttctacgttgactttctgagtcaggacaaggagctgttgccaaagtcttcggccttgttctaccaaaagctgatagaggacaatggctttcctcctttacctgaaaaccagccccttgaagggacatttccctgtgactttgcttggggagttgttgacaactacgttcagctgagtcctttgacaaaacccagtgtcggcctcttgcttcctcactaagggccgcttccctttagtgagggttaatgcttcgagcagacatgataagatacattgatgagtttggacaaaccacaactagaatgcagtgaaaaaaatgctttatttgtgaaatttgtgatgctattgctttatttgtaaccattataagctgcaataaacaagttaacaacaacaattgcattcattttatgtttcaggttcagggggagatgtgggaggttttttaaagcaagtaaaacctctacaaatgtggtaaaatccgataagggactagagcatggctacgtagataagtagcatggcgggttaatcattaactacaaggaacccctagtgatggagttggccactccctctctgcgcgctcgctcgctcactgaggccgggcgaccaaaggtcgcccgacgcccgggctttgcccgggcggcctcagtgagcgagcgagcgcgccagctggcgtaatagcgaagaggcccgcaccgatcgcccttcccaacagttgcgcagcctgaatggcgaatggaattccagacgattgagcgtcaaaatgtaggtatttccatgagcgtttttccgttgcaatggctggcggtaatattgttctggatattaccagcaaggccgatagtttgagttcttctactcaggcaagtgatgttattactaatcaaagaagtattgcgacaacggttaatttgcgtgatggacagactcttttactcggtggcctcactgattataaaaacacttctcaggattctggcgtaccgttcctgtctaaaatccctttaatcggcctcctgtttagctcccgctctgattctaacgaggaaagcacgttatacgtgctcgtcaaagcaaccatagtacgcgccctgtagcggcgcattaagcgcggcgggtgtggtggttacgcgcagcgtgaccgctacacttgccagcgccctagcgcccgctcctttcgctttcttcccttcctttctcgccacgttcgccggctttccccgtcaagctctaaatcgggggctccctttagggttccgatttagtgctttacggcacctcgaccccaaaaaacttgattagggtgatggttcacgtagtgggccatcgccctgatagacggtttttcgccctttgacgttggagtccacgttctttaatagtggactcttgttccaaactggaacaacactcaaccctatctcggtctattcttttgatttataagggattttgccgatttcggcctattggttaaaaaatgagctgatttaacaaaaatttaacgcgaattttaacaaaatattaacgtctacaatttaaatatttgcttatacaatcttcctgtttttggggcttttctgattatcaaccggggtacatatgattgacatgctagttttacgattaccgttcatcgattctcttgtttgctccagactctcaggcaatgacctgatagcctttgtagagacctctcaaaaatagctaccctctccggcatgaatttatcagctagaacggttgaatatcatattgatggtgatttgactgtctccggcctttctcacccgtttgaatctttacctacacattactcaggcattgcatttaaaatatatgagggttctaaaaatttttatccttgcgttgaaataaaggcttctcccgcaaaagtattacagggtcataatgtttttggtacaaccgatttagctttatgctctgaggctttattgcttaattttgctaattctttgccttgcctgtatgatttattggatgttggaatcgcctgatgcggtattttctccttacgcatctgtgcggtatttcacaccgcatatggtgcactctcagtacaatctgctctgatgccgcatagttaagccagccccgacacccgccaacacccgctgacgcgccctgacgggcttgtctgctcccggcatccgcttacagacaagctgtgaccgtctccgggagctgcatgtgtcagaggttttcaccgtcatcaccgaaacgcgcgagacgaaagggcctcgtgatacgcctatttttataggttaatgtcatgataataatggtttcttagacgtcaggtggcacttttcggggaaatgtgcgcggaacccctatttgtttatttttctaaatacattcaaatatgtatccgctcatgagacaataaccctgataaatgcttcaataatattgaaaaaggaagagtatgagtattcaacatttccgtgtcgcccttattcccttttttgcggcattttgccttcctgtttttgctcacccagaaacgctggtgaaagtaaaagatgctgaagatcagttgggtgcacgagtgggttacatcgaactggatctcaacagcggtaagatccttgagagttttcgccccgaagaacgttttccaatgatgagcacttttaaagttctgctatgtggcgcggtattatcccgtattgacgccgggcaagagcaactcggtcgccgcatacactattctcagaatgacttggttgagtactcaccagtcacagaaaagcatcttacggatggcatgacagtaagagaattatgcagtgctgccataaccatgagtgataacactgcggccaacttacttctgacaacgatcggaggaccgaaggagctaaccgcttttttgcacaacatgggggatcatgtaactcgccttgatcgttgggaaccggagctgaatgaagccataccaaacgacgagcgtgacaccacgatgcctgtagcaatggcaacaacgttgcgcaaactattaactggcgaactacttactctagcttcccggcaacaattaatagactggatggaggcggataaagttgcaggaccacttctgcgctcggcccttccggctggctggtttattgctgataaatctggagccggtgagcgtgggtctcgcggtatcattgcagcactggggccagatggtaagccctcccgtatcgtagttatctacacgacggggagtcaggcaactatggatgaacgaaatagacagatcgctgagataggtgcctcactgattaagcattggtaactgtcagaccaagtttactcatatatactttagattgatttaaaacttcatttttaatttaaaaggatctaggtgaagatcctttttgataatctcatgaccaaaatcccttaacgtgagttttcgttccactgagcgtcagaccccgtagaaaagatcaaaggatcttcttgagatcctttttttctgcgcgtaatctgctgcttgcaaacaaaaaaaccaccgctaccagcggtggtttgtttgccggatcaagagctaccaactctttttccgaaggtaactggcttcagcagagcgcagataccaaatactgtccttctagtgtagccgtagttaggccaccacttcaagaactctgtagcaccgcctacatacctcgctctgctaatcctgttaccagtggctgctgccagtggcgataagtcgtgtcttaccgggttggactcaagacgatagttaccggataaggcgcagcggtcgggctgaacggggggttcgtgcacacagcccagcttggagcgaacgacctacaccgaactgagatacctacagcgtgagctatgagaaagcgccacgcttcccgaagggagaaaggcggacaggtatccggtaagcggcagggtcggaacaggagagcgcacgagggagcttccagggggaaacgcctggtatctttatagtcctgtcgggtttcgccacctctgacttgagcgtcgatttttgtgatgctcgtcaggggggcggagcctatggaaaaacgccagcaacgcggcctttttacggttcctggccttttgctggccttttgctcacatgttctttcctgcgttatcccctgattctgtggataaccgtattaccgcctttgagtgagctgataccgctcgccgcagccgaacgaccgagcgcagcgagtcagtgagcgaggaagcggaagagcgcccaatacgcaaaccgcctctccccgcgcgttggccgattcattaatg

SEQ ID NO: 16 - DNA, 18689 bp, Artificial
  Plasmid pXX6
ttattttggattgaagccaatatgataatgagggggtggagtttgtgacgtggcgcggggcgtgggaacggggcgggtgacgtagtagtgtggcggaagtgtgatgttgcaagtgtggcggaacacatgtaagcgacggatgtggcaaaagtgacgtttttggtgtgcgcggatccacaggacgggtgtggtcgccatgatcgcgtagtcgatagtggctccaagtagcgaagcgagcaggactgggcggcggccaaagcggtcggacagtgctccgagaacgggtgcgcatagaaattgcatcaacgcatatagcgctagcagcacgccatagtgactggcgatgctgtcggaatggacgatatcccgcaagaggcccggcagtaccggcataaccaagcctatgcctacagcatccagggtgacggtgccgaggatgacgatgagcgcattgttagatttcatacacggtgcctgactgcgttagcaatttaactgtgataaactaccgcattaaagcttatcgataagcttgatatcgaattcctgcagcccgggggatccactagttctagagcggccgccaccgcggtggagctccaattcgccctatagtgagtcgtattacgcgcgctcactggccgtcgttttacaacgtcgtgactgggaaaaccctggcgttacccaacttaatcgccttgcagcacatccccctttcgccagctggcgtaatagcgaagaggcccgcaccgatcgcccttcccaacagttgcgcagcctgaatggcgaatgggacgcgccctgtagcggcgcattaagcgcggcgggtgtggtggttacgcgcagcgtgaccgctacacttgccagcgccctagcgcccgctcctttcgctttcttcccttcctttctcgccacgttcgccggctttccccgtcaagctctaaatcgggggctccctttagggttccgatttagtgctttacggcacctcgaccccaaaaaacttgattagggtgatggttcacgtagtgggccatcgccctgatagacggtttttcgccctttgacgttggagtccacgttctttaatagtggactcttgttccaaactggaacaacactcaaccctatctcggtctattcttttgatttataagggattttgccgatttcggcctattggttaaaaaatgagctgatttaacaaaaatttaacgcgaattttaacaaaatattaacgcttacaatttaggtggcacttttcggggaaatgtgcgcggaacccctatttgtttatttttctaaatacattcaaatatgtatccgctcatgagacaataaccctgataaatgcttcaataatattgaaaaaggaagagtatgagtattcaacatttccgtgtcgcccttattcccttttttgcggcattttgccttcctgtttttgctcacccagaaacgctggtgaaagtaaaagatgctgaagatcagttgggtgcacgagtgggttacatcgaactggatctcaacagcggtaagatccttgagagttttcgccccgaagaacgttttccaatgatgagcacttttaaagttctgctatgtggcgcggtattatcccgtattgacgccgggcaagagcaactcggtcgccgcatacactattctcagaatgacttggttgagtactcaccagtcacagaaaagcatcttacggatggcatgacagtaagagaattatgcagtgctgccataaccatgagtgataacactgcggccaacttacttctgacaacgatcggaggaccgaaggagctaaccgcttttttgcacaacatgggggatcatgtaactcgccttgatcgttgggaaccggagctgaatgaagccataccaaacgacgagcgtgacaccacgatgcctgtagcaatggcaacaacgttgcgcaaactattaactggcgaactacttactctagcttcccggcaacaattaatagactggatggaggcggataaagttgcaggaccacttctgcgctcggcccttccggctggctggtttattgctgataaatctggagccggtgagcgtgggtctcgcggtatcattgcagcactggggccagatggtaagccctcccgtatcgtagttatctacacgacggggagtcaggcaactatggatgaacgaaatagacagatcgctgagataggtgcctcactgattaagcattggtaactgtcagaccaagtttactcatatatactttagattgatttaaaacttcatttttaatttaaaaggatctaggtgaagatcctttttgataatctcatgaccaaaatcccttaacgtgagttttcgttccactgagcgtcagaccccgtagaaaagatcaaaggatcttcttgagatcctttttttctgcgcgtaatctgctgcttgcaaacaaaaaaaccaccgctaccagcggtggtttgtttgccggatcaagagctaccaactctttttccgaaggtaactggcttcagcagagcgcagataccaaatactgtccttctagtgtagccgtagttaggccaccacttcaagaactctgtagcaccgcctacatacctcgctctgctaatcctgttaccagtggctgctgccagtggcgataagtcgtgtcttaccgggttggactcaagacgatagttaccggataaggcgcagcggtcgggctgaacggggggttcgtgcacacagcccagcttggagcgaacgacctacaccgaactgagatacctacagcgtgagctatgagaaagcgccacgcttcccgaagggagaaaggcggacaggtatccggtaagcggcagggtcggaacaggagagcgcacgagggagcttccagggggaaacgcctggtatctttatagtcctgtcgggtttcgccacctctgacttgagcgtcgatttttgtgatgctcgtcaggggggcggagcctatggaaaaacgccagcaacgcggcctttttacggttcctggccttttgctggccttttgctcacatgttctttcctgcgttatcccctgattctgtggataaccgtattaccgcctttgagtgagctgataccgctcgccgcagccgaacgaccgagcgcagcgagtcagtgagcgaggaagcggaagagcgcccaatacgcaaaccgcctctccccgcgcgttggccgattcattaatgcagctggcacgacaggtttcccgactggaaagcgggcagtgagcgcaacgcaattaatgtgagttagctcactcattaggcaccccaggctttacactttatgcttccggctcgtatgttgtgtggaattgtgagcggataacaatttcacacaggaaacagctatgaccatgattacgccaagcgcgcaattaaccctcactaaagggaacaaaagctgggtaccgggccccccctcgaggtcgacagaagcaccatgtccttgggtccggcctgctgaatgcgcaggcggtcggccatgccccaggcttcgttttgacatcggcgcaggtctttgtagtagtcttgcatgagcctttctaccggcacttcttcttctccttcctcttgtcctgcatctcttgcatctatcgctgcggcggcggcggagtttggccgtaggtggcgccctcttcctcccatgcgtgtgaccccgaagcccctcatcggctgaagcagggctaggtcggcgacaacgcgctcggctaatatggcctgctgcacctgcgtgagggtagactggaagtcatccatgtccacaaagcggtggtatgcgcccgtgttgatggtgtaagtgcagttggccataacggaccagttaacggtctggtgacccggctgcgagagctcggtgtacctgagacgcgagtaagccctcgagtcaaatacgtagtcgttgcaagtccgcaccaggtactggtatcccaccaaaaagtgcggcggcggctggcggtagaggggccagcgtagggtggccggggctccgggggcgagatcttccaacataaggcgatgatatccgtagatgtacctggacatccaggtgatgccggcggcggtggtggaggcgcgcggaaagtcgcggacgcggttccagatgttgcgcagcggcaaaaagtgctccatggtcgggacgctctggccggtcaggcgcgcgcaatcgttgacgctctagcgtgcaaaaggagagcctgtaagcgggcactcttccgtggtctggtggataaattcgcaagggtatcatggcggacgaccggggttcgagccccgtatccggccgtccgccgtgatccatgcggttaccgcccgcgtgtcgaacccaggtgtgcgacgtcagacaacgggggagtgctccttttggcttccttccaggcgcggcggctgctgcgctagcttttttggccactggccgcgcgcagcgtaagcggttaggctggaaagcgaaagcattaagtggctcgctccctgtagccggagggttattttccaagggttgagtcgcgggacccccggttcgagtctcggaccggccggactgcggcgaacgggggtttgcctccccgtcatgcaagaccccgcttgcaaattcctccggaaacagggacgagccccttttttgcttttcccagatgcatccggtgctgcggcagatgcgcccccctcctcagcagcggcaagagcaagagcagcggcagacatgcagggcaccctcccctcctcctaccgcgtcaggaggggcgacatccgcggttgacgcggcagcagatggtgattacgaacccccgcggcgccgggcccggcactacctggacttggaggagggcgagggcctggcgcggctaggagcgccctctcctgagcggtacccaagggtgcagctgaagcgtgatacgcgtgaggcgtacgtgccgcggcagaacctgtttcgcgaccgcgagggagaggagcccgaggagatgcgggatcgaaagttccacgcagggcgcgagctgcggcatggcctgaatcgcgagcggttgctgcgcgaggaggactttgagcccgacgcgcgaaccgggattagtcccgcgcgcgcacacgtggcggccgccgacctggtaaccgcatacgagcagacggtgaaccaggagattaactttcaaaaaagctttaacaaccacgtgcgtacgcttgtggcgcgcgaggaggtggctataggactgatgcatctgtgggactttgtaagcgcgctggagcaaaacccaaatagcaagccgctcatggcgcagctgttccttatagtgcagcacagcagggacaacgaggcattcagggatgcgctgctaaacatagtagagcccgagggccgctggctgctcgatttgataaacatcctgcagagcatagtggtgcaggagcgcagcttgagcctggctgacaaggtggccgccatcaactattccatgcttagcctgggcaagttttacgcccgcaagatataccataccccttacgttcccatagacaaggaggtaaagatcgaggggttctacatgcgcatggcgctgaaggtgcttaccttgagcgacgacctgggcgtttatcgcaacgagcgcatccacaaggccgtgagcgtgagccggcggcgcgagctcagcgaccgcgagctgatgcacagcctgcaaagggccctggctggcacgggcagcggcgatagagaggccgagtcctactttgacgcgggcgctgacctgcgctgggccccaagccgacgcgccctggaggcagctggggccggacctgggctggcggtggcacccgcgcgcgctggcaacgtcggcggcgtggaggaatatgacgaggacgatgagtacgagccagaggacggcgagtactaagcggtgatgtttctgatcagatgatgcaagacgcaacggacccggcggtgcgggcggcgctgcagagccagccgtccggccttaactccacggacgactggcgccaggtcatggaccgcatcatgtcgctgactgcgcgcaatcctgacgcgttccggcagcagccgcaggccaaccggctctccgcaattctggaagcggtggtcccggcgcgcgcaaaccccacgcacgagaaggtgctggcgatcgtaaacgcgctggccgaaaacagggccatccggcccgacgaggccggcctggtctacgacgcgctgcttcagcgcgtggctcgttacaacagcggcaacgtgcagaccaacctggaccggctggtgggggatgtgcgcgaggccgtggcgcagcgtgagcgcgcgcagcagcagggcaacctgggctccatggttgcactaaacgccttcctgagtacacagcccgccaacgtgccgcggggacaggaggactacaccaactttgtgagcgcactgcggctaatggtgactgagacaccgcaaagtgaggtgtaccagtctgggccagactattttttccagaccagtagacaaggcctgcagaccgtaaacctgagccaggctttcaaaaacttgcaggggctgtggggggtgcgggctcccacaggcgaccgcgcgaccgtgtctagcttgctgacgcccaactcgcgcctgttgctgctgctaatagcgcccttcacggacagtggcagcgtgtcccgggacacatacctaggtcacttgctgacactgtaccgcgaggccataggtcaggcgcatgtggacgagcatactttccaggagattacaagtgtcagccgcgcgctggggcaggaggacacgggcagcctggaggcaaccctaaactacctgctgaccaaccggcggcagaagatcccctcgttgcacagtttcgcaccctttggcgcatcccattctccagtaactttatgtccatgggcgcactcacagacctgggccaaaaccttctctacgccaactccgcccacgcgctagacatgacttttgaggtggatcccatggacgagcccacccttctttatgttttgtttgaagtctttgacgtggtccgtgtgcaccggccgcaccgcggcgtcatcgaaaccgtgtacctgcgcacgcccttctcggccggcaacgccacaacataaagaagcaagcaacatcaacaacagctgccgccatgggctccagtgagcaggaactgaaagccattgtcaaagatcttggttgtgggccatattttttgggcacctatgacaagcgctttccaggctttgtttctccacacaagctcgcctgcgccatagtcaatacggccggtcgcgagactgggggcgtacactggatggcctttgcctggaacccgcactcaaaaacatgctacctctttgagccctttggcttttctgaccagcgactcaagcaggtttaccagtttgagtacgagtcactcctgcgccgtagcgccattgcttcttcccccgaccgctgtataacgctggaaaagtccacccaaagcgtacaggggcccaactcggccgcctgtggactattctgctgcatgtttctccacgcctttgccaactggccccaaactcccatggatcacaaccccaccatgaaccttattaccggggtacccaactccatgctcaacagtccccaggtacagcccaccctgcgtcgcaaccaggaacagctctacagcttcctggagcgccactcgccctacttccgcagccacagtgcgcagattaggagcgccacttctttttgtcacttgaaaaacatgtaaaaataatgtactagagacactttcaataaaggcaaatgcttttatttgtacactctcgggtgattatttacccccacccttgccgtctgcgccgtttaaaaatcaaaggggttctgccgcgcatcgctatgcgccactggcagggacacgttgcgatactggtgtttagtgctccacttaaactcaggcacaaccatccgcggcagctcggtgaagttttcactccacaggctgcgcaccatcaccaacgcgtttagcaggtcgggcgccgatatcttgaagtcgcagttggggcctccgccctgcgcgcgcgagttgcgatacacagggttgcagcactggaacactatcagcgccgggtggtgcacgctggccagcacgctcttgtcggagatcagatccgcgtccaggtcctccgcgttgctcagggcgaacggagtcaactttggtagctgccttcccaaaaagggcgcgtgcccaggctttgagttgcactcgcaccgtagtggcatcaaaaggtgaccgtgcccggtctgggcgttaggatacagcgcctgcataaaagccttgatctgcttaaaagccacctgagcctttgcgccttcagagaagaacatgccgcaagacttgccggaaaactgattggccggacaggccgcgtcgtgcacgcagcaccttgcgtcggtgttggagatctgcaccacatttcggccccaccggttcttcacgatcttggccttgctagactgctccttcagcgcgcgctgcccgttttcgctcgtcacatccatttcaatcacgtgctccttatttatcataatgcttccgtgtagacacttaagctcgccttcgatctcagcgcagcggtgcagccacaacgcgcagcccgtgggctcgtgatgcttgtaggtcacctctgcaaacgactgcaggtacgcctgcaggaatcgccccatcatcgtcacaaaggtcttgttgctggtgaaggtcagctgcaacccgcggtgctcctcgttcagccaggtcttgcatacggccgccagagcttccacttggtcaggcagtagtttgaagttcgcctttagatcgttatccacgtggtacttgtccatcagcgcgcgcgcagcctccatgcccttctcccacgcagacacgatcggcacactcagcgggttcatcaccgtaatttcactttccgcttcgctgggctcttcctcttcctcttgcgtccgcataccacgcgccactgggtcgtcttcattcagccgccgcactgtgcgcttacctcctttgccatgcttgattagcaccggtgggttgctgaaacccaccatttgtagcgccacatcttctctttcttcctcgctgtccacgattacctctggtgatggcgggcgctcgggcttgggagaagggcgcttctttttcttcttgggcgcaatggccaaatccgccgccgaggtcgatggccgcgggctgggtgtgcgcggcaccagcgcgtcttgtgatgagtcttcctcgtcctcggactcgatacgccgcctcatccgcttttttgggggcgcccggggaggcggcggcgacggggacggggacgacacgtcctccatggttgggggacgtcgcgccgcaccgcgtccgcgctcgggggtggtttcgcgctgctcctcttcccgactggccatttccttctcctataggcagaaaaagatcatggagtcagtcgagaagaaggacagcctaaccgccccctctgagttcgccaccaccgcctccaccgatgccgccaacgcgcctaccaccttccccgtcgaggcacccccgcttgaggaggaggaagtgattatcgagcaggacccaggttttgtaagcgaagacgacgaggaccgctcagtaccaacagaggataaaaagcaagaccaggacaacgcagaggcaaacgaggaacaagtcgggcggggggacgaaaggcatggcgactacctagatgtgggagacgacgtgctgttgaagcatctgcagcgccagtgcgccattatctgcgacgcgttgcaagagcgcagcgatgtgcccctcgccatagcggatgtcagccttgcctacgaacgccacctattctcaccgcgcgtaccccccaaacgccaagaaaacggcacatgcgagcccaacccgcgcctcaacttctaccccgtatttgccgtgccagaggtgcttgccacctatcacatctttttccaaaactgcaagatacccctatcctgccgtgccaaccgcagccgagcggacaagcagctggccttgcggcagggcgctgtcatacctgatatcgcctcgctcaacgaagtgccaaaaatctttgagggtcttggacgcgacgagaagcgcgcggcaaacgctctgcaacaggaaaacagcgaaaatgaaagtcactctggagtgttggtggaactcgagggtgacaacgcgcgcctagccgtactaaaacgcagcatcgaggtcacccactttgcctacccggcacttaacctaccccccaaggtcatgagcacagtcatgagtgagctgatcgtgcgccgtgcgcagcccctggagagggatgcaaatttgcaagaacaaacagaggagggcctacccgcagttggcgacgagcagctagcgcgctggcttcaaacgcgcgagcctgccgacttggaggagcgacgcaaactaatgatggccgcagtgctcgttaccgtggagcttgagtgcatgcagcggttctttgctgacccggagatgcagcgcaagctagaggaaacattgcactacacctttcgacagggctacgtacgccaggcctgcaagatctccaacgtggagctctgcaacctggtctcctaccttggaattttgcacgaaaaccgccttgggcaaaacgtgcttcattccacgctcaagggcgaggcgcgccgcgactacgtccgcgactgcgtttacttatttctatgctacacctggcagacggccatgggcgtttggcagcagtgcttggaggagtgcaacctcaaggagctgcagaaactgctaaagcaaaacttgaaggacctatggacggccttcaacgagcgctccgtggccgcgcacctggcggacatcattttccccgaacgcctgcttaaaaccctgcaacagggtctgccagacttcaccagtcaaagcatgttgcagaactttaggaactttatcctagagcgctcaggaatcttgcccgccacctgctgtgcacttcctagcgactttgtgcccattaagtaccgcgaatgccctccgccgctttggggccactgctaccttctgcagctagccaactaccttgcctaccactctgacataatggaagacgtgagcggtgacggtctactggagtgtcactgtcgctgcaacctatgcaccccgcaccgctccctggtttgcaattcgcagctgcttaacgaaagtcaaattatcggtacctttgagctgcagggtccctcgcctgacgaaaagtccgcggctccggggttgaaactcactccggggctgtggacgtcggcttaccttcgcaaatttgtacctgaggactaccacgcccacgagattaggttctacgaagaccaatcccgcccgccaaatgcggagcttaccgcctgcgtcattacccagggccacattcttggccaattgcaagccatcaacaaagcccgccaagagtttctgctacgaaagggacggggggtttacttggacccccagtccggcgaggagctcaacccaatccccccgccgccgcagccctatcagcagcagccgcgggcccttgcttcccaggatggcacccaaaaagaagctgcagctgccgccgccacccacggacgaggaggaatactgggacagtcaggcagaggaggttttggacgaggaggaggaggacatgatggaagactgggagagcctagacgaggaagcttccgaggtcgaagaggtgtcagacgaaacaccgtcaccctcggtcgcattcccctcgccggcgccccagaaatcggcaaccggttccagcatggctacaacctccgctcctcaggcgccgccggcactgcccgttcgccgacccaaccgtagatgggacaccactggaaccagggccggtaagtccaagcagccgccgccgttagcccaagagcaacaacagcgccaaggctaccgctcatggcgcgggcacaagaacgccatagttgcttgcttgcaagactgtgggggcaacatctccttcgcccgccgctttcttctctaccatcacggcgtggccttcccccgtaacatcctgcattactaccgtcatctctacagcccatactgcaccggcggcagcggcagcggcagcaacagcagcggccacacagaagcaaaggcgaccggatagcaagactctgacaaagcccaagaaatccacagcggcggcagcagcaggaggaggagcgctgcgtctggcgcccaacgaacccgtatcgacccgcgagcttagaaacaggatttttcccactctgtatgctatatttcaacagagcaggggccaagaacaagagctgaaaataaaaaacaggtctctgcgatccctcacccgcagctgcctgtatcacaaaagcgaagatcagcttcggcgcacgctggaagacgcggaggctctcttcagtaaatactgcgcgctgactcttaaggactagtttcgcgccctttctcaaatttaagcgcgaaaactacgtcatctccagcggccacacccggcgccagcacctgtcgtcagcgccattatgagcaaggaaattcccacgccctacatgtggagttaccagccacaaatgggacttgcggctggagctgcccaagactactcaacccgaataaactacatgagcgcgggaccccacatgatatcccgggtcaacggaatccgcgcccaccgaaaccgaattctcttggaacaggcggctattaccaccacacctcgtaataaccttaatccccgtagttggcccgctgccctggtgtaccaggaaagtcccgctcccaccactgtggtacttcccagagacgcccaggccgaagttcagatgactaactcaggggcgcagcttgcgggcggctttcgtcacagggtgcggtcgcccgggcagggtataactcacctgacaatcagagggcgaggtattcagctcaacgacgagtcggtgagctcctcgcttggtctccgtccggacgggacatttcagatcggcggcgccggccgtccttcattcacgcctcgtcaggcaatcctaactctgcagacctcgtcctctgagccgcgctctggaggcattggaactctgcaatttattgaggagtttgtgccatcggtctactttaaccccttctcgggacctcccggccactatccggatcaatttattcctaactttgacgcggtaaaggactcggcggacggctacgactgaatgttaagtggagaggcagagcaactgcgcctgaaacacctggtccactgtcgccgccacaagtgctttgcccgcgactccggtgagttttgctactttgaattgcccgaggatcatatcgagggcccggcgcacggcgtccggcttaccgcccagggagagcttgcccgtagcctgattcgggagtttacccagcgccccctgctagttgagcgggacaggggaccctgtgttctcactgtgatttgcaactgtcctaaccttggattacatcaaccctttaactaataaaaaaaaataataaagcatcacttacttaaaatcagttagcaaatttctgtccagtttattcagcagcacctccttgccctcctcccagctctggtattgcagcttcctcctggctgcaaactttctccacaatctaaatggaatgtcagtttcctcctgttcctgtccatccgcacccactatcttcatgttgttgcagatgaagcgcgcaagaccgtctgaagataccttcaaccccgtgtatccatatgacacggaaaccggtcctccaactgtgccttttcttactcctccctttgtatcccccaatgggtttcaagagagtccccctggggtactctctttgcgcctatccgaacctctagttacctccaatggcatgcttgcgctcaaaatgggcaacggcctctctctggacgaggccggcaaccttacctcccaaaatgtaaccactgtgagcccacctctcaaaaaaaccaagtcaaacataaacctggaaatatctgcacccctcacagttacctcagaagccctaactgtggctgccgccgcacctctaatggtcgcgggcaacacactcaccatgcaatcacaggccccgctaaccgtgcacgactccaaacttagcattgccacccaaggacccctcacagtgtcagaaggaaagctagccctgcaaacatcaggccccctcaccaccaccgatagcagtacccttactatcactgcctcaccccctctaactactgccactggtagcttgggcattgacttgaaagagcccatttatacacaaaatggaaaactaggactaaagtacggggctcctttgcatgtaacagacgacctaaacactttgaccgtagcaactggtccaggtgtgactattaataatacttccttgcaaactaaagttactggagccttgggttttgattcacaaggcaatatgcaacttaatgtagcaggaggactaaggattgattctcaaaacagacgccttatacttgatgttagttatccgtttgatgctcaaaaccaactaaatctaagactaggacagggccctctttttataaactcagcccacaacttggatattaactacaacaaaggcctttacttgtttacagcttcaaacaattccaaaaagcttgaggttaacctaagcactgccaaggggttgatgtttgacgctacagccatagccattaatgcaggagatgggcttgaatttggttcacctaatgcaccaaacacaaatcccctcaaaacaaaaattggccatggcctagaatttgattcaaacaaggctatggttcctaaactaggaactggccttagttttgacagcacaggtgccattacagtaggaaacaaaaataatgataagctaactttgtggaccacaccagctccatctcctaactgtagactaaatgcagagaaagatgctaaactcactttggtcttaacaaaatgtggcagtcaaatacttgctacagtttcagttttggctgttaaaggcagtttggctccaatatctggaacagttcaaagtgctcatcttattataagatttgacgaaaatggagtgctactaaacaattccttcctggacccagaatattggaactttagaaatggagatcttactgaaggcacagcctatacaaacgctgttggatttatgcctaacctatcagcttatccaaaatctcacggtaaaactgccaaaagtaacattgtcagtcaagtttacttaaacggagacaaaactaaacctgtaacactaaccattacactaaacggtacacaggaaacaggagacacaactccaagtgcatactctatgtcattttcatgggactggtctggccacaactacattaatgaaatatttgccacatcctcttacactttttcatacattgcccaagaataaagaatcgtttgtgttatgtttcaacgtgtttatttttcaattgcagaaaatttcaagtcatttttcattcagtagtatagccccaccaccacatagcttatacagatcaccgtaccttaatcaaactcacagaaccctagtattcaacctgccacctccctcccaacacacagagtacacagtcctttctccccggctggccttaaaaagcatcatatcatgggtaacagacatattcttaggtgttatattccacacggtttcctgtcgagccaaacgctcatcagtgatattaataaactccccgggcagctcacttaagttcatgtcgctgtccagctgctgagccacaggctgctgtccaacttgcggttgcttaacgggcggcgaaggagaagtccacgcctacatgggggtagagtcataatcgtgcatcaggatagggcggtggtgctgcagcagcgcgcgaataaactgctgccgccgccgctccgtcctgcaggaatacaacatggcagtggtctcctcagcgatgattcgcaccgcccgcagcataaggcgccttgtcctccgggcacagcagcgcaccctgatctcacttaaatcagcacagtaactgcagcacagcaccacaatattgttcaaaatcccacagtgcaaggcgctgtatccaaagctcatggcggggaccacagaacccacgtggccatcataccacaagcgcaggtagattaagtggcgacccctcataaacacgctggacataaacattacctcttttggcatgttgtaattcaccacctcccggtaccatataaacctctgattaaacatggcgccatccaccaccatcctaaaccagctggccaaaacctgcccgccggctatacactgcagggaaccgggactggaacaatgacagtggagagcccaggactcgtaaccatggatcatcatgctcgtcatgatatcaatgttggcacaacacaggcacacgtgcatacacttcctcaggattacaagctcctcccgcgttagaaccatatcccagggaacaacccattcctgaatcagcgtaaatcccacactgcagggaagacctcgcacgtaactcacgttgtgcattgtcaaagtgttacattcgggcagcagcggatgatcctccagtatggtagcgcgggtttctgtctcaaaaggaggtagacgatccctactgtacggagtgcgccgagacaaccgagatcgtgttggtcgtagtgtcatgccaaatggaacgccggacgtagtcatatttcctgaagcaaaaccaggtgcgggcgtgacaaacagatctgcgtctccggtctcgccgcttagatcgctctgtgtagtagttgtagtatatccactctctcaaagcatccaggcgccccctggcttcgggttctatgtaaactccttcatgcgccgctgccctgataacatccaccaccgcagaataagccacacccagccaacctacacattcgttctgcgagtcacacacgggaggagcgggaagagctggaagaaccatgtttttttttttattccaaaagattatccaaaacctcaaaatgaagatctattaagtgaacgcgctcccctccggtggcgtggtcaaactctacagccaaagaacagataatggcatttgtaagatgttgcacaatggcttccaaaaggcaaacggccctcacgtccaagtggacgtaaaggctaaacccttcagggtgaatctcctctataaacattccagcaccttcaaccatgcccaaataattctcatctcgccaccttctcaatatatctctaagcaaatcccgaatattaagtccggccattgtaaaaatctgctccagagcgccctccaccttcagcctcaagcagcgaatcatgattgcaaaaattcaggttcctcacagacctgtataagattcaaaagcggaacattaacaaaaataccgcgatcccgtaggtcccttcgcagggccagctgaacataatcgtgcaggtctgcacggaccagcgcggccacttccccgccaggaaccttgacaaaagaacccacactgattatgacacgcatactcggagctatgctaaccagcgtagccccgatgtaagctttgttgcatgggcggcgatataaaatgcaaggtgctgctcaaaaaatcaggcaaagcctcgcgcaaaaaagaaagcacatcgtagtcatgctcatgcagataaaggcaggtaagctccggaaccaccacagaaaaagacaccatttttctctcaaacatgtctgcgggtttctgcataaacacaaaataaaataacaaaaaaacatttaaacattagaagcctgtcttacaacaggaaaaacaacccttataagcataagacggactacggccatgccggcgtgaccgtaaaaaaactggtcaccgtgattaaaaagcaccaccgacagctcctcggtcatgtccggagtcataatgtaagactcggtaaacacatcaggttgattcatcggtcagtgctaaaaagcgaccgaaatagcccgggggaatacatacccgcaggcgtagagacaacattacagcccccataggaggtataacaaaattaataggagagaaaaacacataaacacctgaaaaaccctcctgcctaggcaaaatagcaccctcccgctccagaacaacatacagcgcttcacagcggcagcctaacagtcagccttaccagtaaaaaagaaaacctattaaaaaaacaccactcgacacggcaccagctcaatcagtcacagtgtaaaaaagggccaagtgcagagcgagtatatataggactaaaaaatgacgtaacggttaaagtccacaaaaaacacccagaaaaccgcacgcgaacctacgcccagaaacgaaagccaaaaaacccacaacttcctcaaatcgtcacttccgttttcccacgttacgtaacttcccattttaagaaaactacaattcccaacacatacaagttactccgccctaaaacctacgtcacccgccccgttcccacgccccgcgccacgtcacaaactccaccccctcattatcatattggcttcaatccaaaataaggtatattattgatgatg

SEQ ID NO: 17 - DNA, 7335 bp, Artificial
  Plasmid pREp2Cap10
gattaaggtccccagcgaccttgacgagcatctgcccggcatttctgacagctttgtgaactgggtggccgagaaggaatgggagttgccgccagattctgacatggatctgaatctgattgagcaggcacccctgaccgtggccgagaagctgcagcgcgactttctgacggaatggcgccgtgtgagtaaggccccggaggctcttttctttgtgcaatttgagaagggagagagctacttccacatgcacgtgctcgtggaaaccaccggggtgaaatccatggttttgggacgtttcctgagtcagattcgcgaaaaactgattcagagaatttaccgcgggatcgagccgactttgccaaactggttcgcggtcacaaagaccagaaatggcgccggaggcgggaacaaggtggtggatgagtgctacatccccaattacttgctccccaaaacccagcctgagctccagtgggcgtggactaatatggaacagtatttaagcgcctgtttgaatctcacggagcgtaaacggttggtggcgcagcatctgacgcacgtgtcgcagacgcaggagcagaacaaagagaatcagaatcccaattctgatgcgccggtgatcagatcaaaaacttcagccaggtacatggagctggtcgggtggctcgtggacaaggggattacctcggagaagcagtggatccaggaggaccaggcctcatacatctccttcaatgcggcctccaactcgcggtcccaaatcaaggctgccttggacaatgcgggaaagattatgagcctgactaaaaccgcccccgactacctggtgggccagcagcccgtggaggacatttccagcaatcggatttataaaattttggaactaaacgggtacgatccccaatatgcggcttccgtctttctgggatgggccacgaaaaagttcggcaagaggaacaccatctggctgtttgggcctgcaactaccgggaagaccaacatcgcggaggccatagcccacactgtgcccttctacgggtgcgtaaactggaccaatgagaactttcccttcaacgactgtgtcgacaagatggtgatctggtgggaggaggggaagatgaccgccaaggtcgtggagtcggccaaagccattctcggaggaagcaaggtgcgcgtggaccagaaatgcaagtcctcggcccagatagacccgactcccgtgatcgtcacctccaacaccaacatgtgcgccgtgattgacgggaactcaacgaccttcgaacaccagcagccgttgcaagaccggatgttcaaatttgaactcacccgccgtctggatcatgactttgggaaggtcaccaagcaggaagtcaaagactttttccggtgggcaaaggatcacgtggttgaggtggagcatgaattctacgtcaaaaagggtggagccaagaaaagacccgcccccagtgacgcagatataagtgagcccaaacgggtgcgcgagtcagttgcgcagccatcgacgtcagacgcggaagcttcgatcaactacgcagacaggtaccaaaacaaatgttctcgtcacgtgggcatgaatctgatgctgtttccctgcagacaatgcgagagaatgaatcagaattcaaatatctgcttcactcacggacagaaagactgtttagagtgctttcccgtgtcagaatctcaacccgtttctgtcgtcaaaaaggcgtatcagaaactgtgctacattcatcatatcatgggaaaggtgccagacgcttgcactgcctgcgatctggtcaatgtggatttggatgactgcatctttgaacaataaatgatttaaatcaggtatggctgccgatggttatcttccagattggctcgaggacaacctctctgagggcattcgcgagtggtgggacttgaaacctggagccccgaaacccaaagccaaccagcaaaagcaggacgacggccggggtctggtgcttcctggctacaagtacctcggacccttcaacggactcgacaagggggagcccgtcaacgcggcggacgcagcggccctcgagcacgacaaggcctacgaccagcagctcaaagcgggtgacaatccgtacctgcggtataaccacgccgacgccgagtttcaggagcgtctgcaagaagatacgtcttttgggggcaacctcgggcgagcagtcttccaggccaagaagcgggttctcgaacctctcggtctggttgaggaaggcgctaagacggctcctggaaagaagagaccggtagagccatcaccccagcgttctccagactcctctacgggcatcggcaagaaaggccagcagcccgcgaaaaagagactcaactttgggcagactggcgactcagagtcagtgcccgaccctcaaccaatcggagaaccccccgcaggcccctctggtctgggatctggtacaatggctgcaggcggtggcgctccaatggcagacaataacgaaggcgccgacggagtgggtagttcctcaggaaattggcattgcgattccacatggctgggcgacagagtcatcaccaccagcacccgaacctgggccctccccacctacaacaaccacctctacaagcaaatctccaacgggacttcgggaggaagcaccaacgacaacacctacttcggctacagcaccccctgggggtattttgactttaacagattccactgccacttctcaccacgtgactggcagcgactcatcaacaacaactggggattccggcccaagagactcaacttcaagctcttcaacatccaggtcaaggaggtcacgcagaatgaaggcaccaagaccatcgccaataaccttaccagcacgattcaggtctttacggactcggaataccagctcccgtacgtcctcggctctgcgcaccagggctgcctgcctccgttcccggcggacgtcttcatgattcctcagtacgggtacctgactctgaacaatggcagtcaggccgtgggccgttcctccttctactgcctggagtactttccttctcaaatgctgagaacgggcaacaactttgagttcagctaccagtttgaggacgtgccttttcacagcagctacgcgcacagccaaagcctggaccggctgatgaaccccctcatcgaccagtacctgtactacctgtctcggactcagtccacgggaggtaccgcaggaactcagcagttgctattttctcaggccgggcctaataacatgtcggctcaggccaaaaactggctacccgggccctgctaccggcagcaacgcgtctccacgacactgtcgcaaaataacaacagcaactttgcctggaccggtgccaccaagtatcatctgaatggcagagactctctggtaaatcccggtgtcgctatggcaacccacaaggacgacgaagagcgattttttccgtccagcggagtcttaatgtttgggaaacagggagctggaaaagacaacgtggactatagcagcgttatgctaaccagtgaggaagaaattaaaaccaccaacccagtggccacagaacagtacggcgtggtggccgataacctgcaacagcaaaacgccgctcctattgtaggggccgtcaacagtcaaggagccttacctggcatggtctggcagaaccgggacgtgtacctgcagggtcctatctgggccaagattcctcacacggacggaaactttcatccctcgccgctgatgggaggctttggactgaaacacccgcctcctcagatcctgattaagaatacacctgttcccgcggatcctccaactaccttcagtcaagctaagctggcgtcgttcatcacgcagtacagcaccggacaggtcagcgtggaaattgaatgggagctgcagaaagaaaacagcaaacgctggaacccagagattcaatacacttccaactactacaaatctacaaatgtggactttgctgttaacacagatggcacttattctgagcctcgccccatcggcacccgttacctcacccgtaatctgtaattgcttgttaatcaataaaccggttgattcgtttcagttgaactttggtctctgcatatggcgaattcgtttaaacctgcaggactagagtcctgtattagaggtcacgtgagtgttttgcgacattttgcgacaccatgtggtcacgctgggtatttaagcccgagtgagcacgcagggtctccattttgaagcgggaggtttgaacgcgcagccgccaagccgaattctgcagatatccatcacactggcggccgctcgactagagcggccgccaccgcggtggagctccagcttttgttccctttagtgagggttaattgcgcgcttggcgtaatcatggtcatagctgtttcctgtgtgaaattgttatccgctcacaattccacacaacatacgagccggaagcataaagtgtaaagcctggggtgcctaatgagtgagctaactcacattaattgcgttgcgctcactgcccgctttccagtcgggaaacctgtcgtgccagctgcattaatgaatcggccaacgcgcggggagaggcggtttgcgtattgggcgctcttccgcttcctcgctcactgactcgctgcgctcggtcgttcggctgcggcgagcggtatcagctcactcaaaggcggtaatacggttatccacagaatcaggggataacgcaggaaagaacatgtgagcaaaaggccagcaaaaggccaggaaccgtaaaaaggccgcgttgctggcgtttttccataggctccgcccccctgacgagcatcacaaaaatcgacgctcaagtcagaggtggcgaaacccgacaggactataaagataccaggcgtttccccctggaagctccctcgtgcgctctcctgttccgaccctgccgcttaccggatacctgtccgcctttctcccttcgggaagcgtggcgctttctcatagctcacgctgtaggtatctcagttcggtgtaggtcgttcgctccaagctgggctgtgtgcacgaaccccccgttcagcccgaccgctgcgccttatccggtaactatcgtcttgagtccaacccggtaagacacgacttatcgccactggcagcagccactggtaacaggattagcagagcgaggtatgtaggcggtgctacagagttcttgaagtggtggcctaactacggctacactagaagaacagtatttggtatctgcgctctgctgaagccagttaccttcggaaaaagagttggtagctcttgatccggcaaacaaaccaccgctggtagcggtggtttttttgtttgcaagcagcagattacgcgcagaaaaaaaggatctcaagaagatcctttgatcttttctacggggtctgacgctcagtggaacgaaaactcacgttaagggattttggtcatgagattatcaaaaaggatcttcacctagatccttttaaattaaaaatgaagttttaaatcaatctaaagtatatatgagtaaacttggtctgacagttaccaatgcttaatcagtgaggcacctatctcagcgatctgtctatttcgttcatccatagttgcctgactccccgtcgtgtagataactacgatacgggagggcttaccatctggccccagtgctgcaatgataccgcgagacccacgctcaccggctccagatttatcagcaataaaccagccagccggaagggccgagcgcagaagtggtcctgcaactttatccgcctccatccagtctattaattgttgccgggaagctagagtaagtagttcgccagttaatagtttgcgcaacgttgttgccattgctacaggcatcgtggtgtcacgctcgtcgtttggtatggcttcattcagctccggttcccaacgatcaaggcgagttacatgatcccccatgttgtgcaaaaaagcggttagctccttcggtcctccgatcgttgtcagaagtaagttggccgcagtgttatcactcatggttatggcagcactgcataattctcttactgtcatgccatccgtaagatgcttttctgtgactggtgagtactcaaccaagtcattctgagaatagtgtatgcggcgaccgagttgctcttgcccggcgtcaatacgggataataccgcgccacatagcagaactttaaaagtgctcatcattggaaaacgttcttcggggcgaaaactctcaaggatcttaccgctgttgagatccagttcgatgtaacccactcgtgcacccaactgatcttcagcatcttttactttcaccagcgtttctgggtgagcaaaaacaggaaggcaaaatgccgcaaaaaagggaataagggcgacacggaaatgttgaatactcatactcttcctttttcaatattattgaagcatttatcagggttattgtctcatgagcggatacatatttgaatgtatttagaaaaataaacaaataggggttccgcgcacatttccccgaaaagtgccacctaaattgtaagcgttaatattttgttaaaattcgcgttaaatttttgttaaatcagctcattttttaaccaataggccgaaatcggcaaaatcccttataaatcaaaagaatagaccgagatagggttgagtgttgttccagtttggaacaagagtccactattaaagaacgtggactccaacgtcaaagggcgaaaaaccgtctatcagggcgatggcccactacgtgaaccatcaccctaatcaagttttttggggtcgaggtgccgtaaagcactaaatcggaaccctaaagggagcccccgatttagagcttgacggggaaagccggcgaacgtggcgagaaaggaagggaagaaagcgaaaggagcgggcgctagggcgctggcaagtgtagcggtcacgctgcgcgtaaccaccacacccgccgcgcttaatgcgccgctacagggcgcgtcccattcgccattcaggctgcgcaactgttgggaagggcgatcggtgcgggcctcttcgctattacgccagctggcgaaagggggatgtgctgcaaggcgattaagttgggtaacgccagggttttcccagtcacgacgttgtaaaacgacggccagtgagcgcgcgtaatacgactcactatagggcgaattgggtaccgggccccccctcgatcgaggtcgacggtatcgggggagctcgcagggtctccattttgaagcgggaggtttgaacgcgcagccgccatgccggggttttacgagattgt

SEQ ID NO: 18 - DNA, 22 bp, Artificial
  Forward primer
tacataacttacggtaaatggc

SEQ ID NO: 19 - DNA, 21 bp, Artificial
  Reverse primer
aaagtccctattggcgttact